European Patent Application EP 4 725 551 A1, published April 15, 2026. Title: FUSION POLYPEPTIDE AJ007 AND USE THEREOF. Applicant: Nanjing Anji Biotechnology CO., LTD. Application EP. The sequence listing filed with the application follows.

SEQUENCE LISTING (2 sequences)

SEQ ID NO: 1 - protein, 13 aa, synthetic construct
RGADRAGGGGRGD

SEQ ID NO: 2 - protein, 24 aa, synthetic construct
YGRKKRRQRRRRGADRAGGGGRGD